European Patent Specification EP 3 877 402 B1, published July 16, 2025. Title: COMBINATION TREATMENT FOR RESISTANT HYPERTENSION. Applicant: Mayo Foundation for Medical Education and Research. The sequence listing filed with the application follows.

SEQUENCE LISTING (14 sequences)

SEQ ID NO: 1 - protein, 28 aa, Homo sapiens
SLRRSSCFGGRMDRIGAQSGLGCNSFRY

SEQ ID NO: 2 - protein, 12 aa, Homo sapiens
RITAREDKQGWA

SEQ ID NO: 3 - protein, 40 aa, Homo sapiens
SLRRSSCFGGRMDRIGAQSGLGCNSFRYRITAREDKQGWA

SEQ ID NO: 4 - DNA, 123 bp, Homo sapiens
agcctgcggagatccagctgcttcgggggcaggatggacaggattggagcccagagcggactgggctgtaacagcttccggtaccggataacagccagggaggacaagcagggctgggcctag

SEQ ID NO: 5 - protein, 39 aa, Artificial Sequence
  synthetic
SLRRSSCFGGRMDRIGAQSGLGCNSFRYRIAREDKQGWA

SEQ ID NO: 6 - protein, 40 aa, Artificial
  synthetic
SLRRSSCFGGRMDRIGAQSGLGCNSFRYRITAREDKQGYA

SEQ ID NO: 7 - protein, 41 aa, Artificial Sequence
  synthetic
SLRRSSCFGGRMDRIGAQSGLGCNSFRYRITAREDKSQGWA

SEQ ID NO: 8 - protein, 37 aa, Artificial Sequence
  synthetic
SLRRSSCFGGRMDRIGAQSGLGCNSFRYRITAREDKQ

SEQ ID NO: 9 - protein, 44 aa, Artificial Sequence
  synthetic
TAPRSLRRSSCFGGRMDRIGAQSGLGCNSFRYRITAREDKQGWA

SEQ ID NO: 10 - protein, 40 aa, Artificial Sequence
  synthetic
SLKKSSCFGGRMDRIGAQSGLGCNSFRYRITAREDKQGWA

SEQ ID NO: 11 - protein, 40 aa, Artificial Sequence; identical to SEQ ID NO: 3
  synthetic
  MISC_FEATURE (6)..(6): Ser is D-isoform

SEQ ID NO: 12 - protein, 39 aa, Artificial Sequence
  synthetic
  MISC_FEATURE (4)..(4): Arg is D-isoform
SLRRSCFGGRMDRIGAQSGLGCNSFRYRITAREDKQGWA

SEQ ID NO: 13 - protein, 40 aa, Artificial Sequence
  synthetic
TLRRTTCFGGRMDRIGAQSGLGCNSFRYRITAREDKQGWA

SEQ ID NO: 14 - protein, 40 aa, Artificial  Sequence
  synthetic
SWRRSSCFGGRMDRIGAQSGLGCNSFRYRITAREDKQGWA